European Patent Specification EP 3 645 730 B1, published July 31, 2024. Title: Utilisation des polykétide synthases de type III comme phloroglucinol synthases. Applicant: COMPAGNIE GENERALE DES ETABLISSEMENTS MICHELIN. The sequence listing filed with the application follows.

SEQUENCE LISTING (9 sequences)

SEQ ID NO: 1 - protein, 413 aa, Sargassum binderi
MSSAAVAMLADPTVQIALACIVLSLIVVFRSYRKGKDEQTVYPVIAGMAIGNPQYRCTQDQALTVAQKCPGVESVKPVLERIYGNSRIGSRYFAVPDFTPNQAAKGDPMFFPADGSFEVPVDTRLDKFKEKAVPLVSDVARRAIKEAGIDVSDVSKLVVVSSTGFLGPGLDCELIKNLGLTRSVDRTLIGFMGCAAAMNGFRNANDFVTANPGKYALMICVELSSVHTTFDDNINDAILHAIFADGCAAAVLKGVRKEAPKGTLAIVDNHAWLMEGTEDGITLAIKPNGITCTLSKFLPQYIAKNIAFFADGFLKKHNLGRDDVDFWCVHPGGRRIIEEAQNGLGLTEAQTADSWAVLAEYGNMLSPSVMFVLSRVFKRHNAALAQGKPGYQTGMAFSFSPGVGAEGILLRQI

SEQ ID NO: 2 - protein, 297 aa, Aureococcus anophagefferens
MPVEKRLDMFREKSVPLVTKVCKDAMADAGIDVEQIGKLVVVSSTGFLGPGLDAELIKTLGLWRGVDRSLIGFMGCAAAMNGFRVANDFAMSHPGKMALMVCVEISSVHTTFDDNVNDAILHAIFADGCAAAVISGEKPGSAAAKGKFGIVDTHGWLMEGTEDGITLSINENGISCILSKYLPQYIAKNMAGYVDSFLGMHGLQKTDMDFWAIHPGGRRIIEEAQNGLGLSEEQAKYSWTVLSQYGNMLSPSVMFVLELILNDHKKALAKGERGLKQGIAFSFSPGVGAEGILINVM

SEQ ID NO: 3 - protein, 382 aa, Aureococcus anophagefferens
MSKKDEKIIPVIMGMATGNPPYRASQQQALAIAESCPECNSIKPVLARIYGNSRIDYRFMAVPDFTPEQKLEGDENFFDKDLMFKMPVEKRLDMFREKSVPLVTKVCKDAMADAGIDVEQIGKLVVVSSTGFLGPGLDAELIKTLGLWRGVDRSLIGFMGCAAAMNGFRVANDFAMSHPGKMALMVCVEISSVHTTFDDNVNDAILHAIFADGCAAAVISGEKPGSAAAKGKFGIVDTHGWLMEGTEDGITLSINENGISCILSKYLPQYIAKNMAGYVDSFLGMHGLQKTDMDFWAIHPGGRRIIEEAQNGLGLSEEQAKYSWTVLSQYGNMLSPSVMFVLELILNDHKKALAKGERGLKQGIAFSFSPGVGAEGILINVM

SEQ ID NO: 4 - DNA, 1149 bp, Aureococcus anophagefferens
atgtcgaagaaggatgagaagatcatccctgtcatcatgggtatggccacaggtaatccgccatacagggcgagtcaacaacaagctctagcaattgcggagtcctgcccagaatgtaatagcattaaaccggtattggcaagaatttatggtaatagccgtatcgactacaggtttatggcagtaccggatttcacacccgaacagaagcttgaaggtgacgaaaacttctttgataaagatttaatgtttaagatgccagtggagaagagattggacatgtttagggagaagagtgtgccattagtcacgaaggtctgtaaggatgccatggcagacgctggtatagacgttgaacagattggcaaacttgtcgtggtatcatcaactggcttcttaggccctggactagatgcggagttaattaagacacttggactttggcgtggtgttgaccggtctctgattggattcatgggttgtgcggcggccatgaacggttttcgggttgctaatgatttcgccatgtcccacccgggaaagatggccctaatggtttgcgtcgaaatatcctctgtgcataccacattcgatgataacgtaaatgatgcaatacttcatgcgatcttcgccgatggatgtgcagccgcagtaatatcgggagagaagccaggttctgcggcagcgaaaggcaaattcggaatcgtcgatacgcatggttggctcatggaaggcacagaagatgggataaccctgtctatcaatgaaaatggtatatcatgcatcttgagtaagtatctaccacagtatattgcaaagaacatggcaggttacgtagatagtttcctagggatgcatggattacagaagacagatatggatttctgggctattcaccccggcggccgcagaattatagaggaagcgcagaacggtttgggtttatccgaggagcaggcgaagtattcttggactgttcttagtcagtatggtaatatgttgtcacctagcgtgatgtttgtgttagaactgatccttaatgaccacaagaaggcactggcaaagggagagcgcggtttaaagcaaggtatcgcatttagcttctcaccgggtgttggggccgagggcatcctcattaatgttatgtaa

SEQ ID NO: 5 - protein, 349 aa, Pseudomonas fluorescens Pf5
MSTLCLPHVMFPQHKITQQQMVDHLENLHADHPRMALAKRMIANTEVNERHLVLPIDELAVHTGFTHRSIVYEREARQMSSAAARQAIENAGLQISDIRMVIVTSCTGFMMPSLTAHLINDLALPTSTVQLPIAQLGCVAGAAAINRANDFARLDARNHVLIVSLEFSSLCYQPDDTKLHAFISAALFGDAVSACVLRADDQAGGFKIKKTESYFLPKSEHYIKYDVKDTGFHFTLDKAVMNSIKDVAPVMERLNYESFEQNCAHNDFFIFHTGGRKILDELVMHLDLASNRVSQSRSSLSEAGNIASVVVFDVLKRQFDSNLNRGDIGLLAAFGPGFTAEMAVGEWTA

SEQ ID NO: 6 - protein, 381 aa, Ectocarpus siliculosus
MSKDEQTVYPVIAGMAIGNPQYRCTQNEALAVASKCPGLESIKPVLERIYGNSRIGSRYFAVPDFTPGRAAKGDPLFYPADGSYQVPVDVRLDKFKEKAVPLVSDVARRAIKEAGLNVEDISKLVVVSSTGFLGPGLDCELIKNLGLTRSVDRTLIGFMGCAAAMNGFRNANDYVTANPGKYALMICVELSSVHTTFDDNINDAILHAIFADGCAAAVLKGARKSECPKGTLAIVDNHAWLMEGTEDGITLAIKPNGITCTLSKFLPQYIAKNIAFFADGFLKKHKLGRDDVDFWCVHPGGRRIIEEAQNGLGLSEEQTADSWAVLGEYGNMLSPSVMFVLSRVFKRHNAALAQGKPGYQTGMAFSFSPGVGAEGILLRQI

SEQ ID NO: 7 - DNA, 598 bp, Saccharomyces cerevisiae
tatcttaactgatagtttgatcaaaggggcaaaacgtaggggcaaacaaacggaaaaatcgtttctcaaattttctgatgccaagaactctaaccagtcttatctaaaaattgccttatgatccgtctctccggttacagcctgtgtaactgattaatcctgcctttctaatcaccattctaatgttttaattaagggattttgtcttcattaacggctttcgctcataaaaatgttatgacgttttgcccgcaggcgggaaaccatccacttcacgagactgatctcctctgccggaacaccgggcatctccaacttataagttggagaaataagagaatttcagattgagagaatgaaaaaaaaaaaaaaaaaaggcagaggagagcatagaaatggggttcactttttggtaaagctatagcatgcctatcacatataaatagagtgccagtagcgacttttttcacactcgaaatactcttactactgctctcttgttgtttttatcacttcttgtttcttcttggtaaatagaatatcaagctacaaaaagcatacaatcaactatcaactattaactatatcgtaatacaca

SEQ ID NO: 8 - DNA, 998 bp, Saccharomyces cerevisiae
aaccagggcaaagcaaaataaaagaaacttaatacgttatgccgtaatgaagggctaccaaaaacgataatctcaactgtaaacaggtacaatgcggacccttttgccacaaaacatacatcattcattgccggaaaaagaaagaagtgaagacagcagtgcagccagccatgttgcgccaatctaattatagatgctggtgccctgaggatgtatctggagccagccatggcatcatgcgctaccgccggatgtaaaatccgacacgcaaaagaaaaccttcgaggttgcgcacttcgcccacccatgaaccacacggttagtccaaaaggggcagttcagattccagatgcgggaattagcttgctgccaccctcacctcactaacgctgcggtgtgcggatacttcatgctatttatagacgcgcgtgtcggaatcagcacgcgcaagaaccaaatgggaaaatcggaatgggtccagaactgctttgagtgctggctattggcgtctgatttccgttttgggaatcctttgccgcgcgcccctctcaaaactccgcacaagtcccagaaagcgggaaagaaataaaacgccaccaaaaaaaaaaataaaagccaatcctcgaagcgtgggtggtaggccctggattatcccgtacaagtatttctcaggagtaaaaaaaccgtttgttttggaattccccatttcgcggccacctacgccgctatctttgcaacaactatctgcgataactcagcaaattttgcatattcgtgttgcagtattgcgataatgggagtcttacttccaacataacggcagaaagaaatgtgagaaaattttgcatcctttgcctccgttcaagtatataaagtcggcatgcttgataatctttctttccatcctacattgttctaattattcttattctcctttattctttcctaacataccaagaaattaatcttctgtcattcgcttaaacactatatcaata

SEQ ID NO: 9 - DNA, 300 bp, Saccharomyces cerevisiae
gaagttttgttagaaaataaatcattttttaattgagcattcttattcctattttatttaaatagttttatgtattgttagctacatacaacagtttaaatcaaattttctttttcccaagtccaaaatggaggtttattttgatgacccgcatgcgattatgttttgaaagtataagactacatacatgtacatatatttaaacatgtaaacccgtccattatattgcttactttcttcttttttgccgttttgacttggacctctggtttgctatttccttacaatctttgctacaat